European Patent Application EP 4 575 001 A1, published June 25, 2025. Title: A METHOD OF GENOTYPING SINGLE NUCLEOTIDE POLYMORPHISMS THAT ARE ASSOCIATED WITH THE PRODUCTION AND QUALITY OF SHEEP MILK. Applicant: INSTITUTO NACIONAL DE INVESTIGAÇÃO AGRÁRIA E VETERINÁRIA, I.P. Application PT N/A. The sequence listing filed with the application follows.

SEQUENCE LISTING (36 sequences)

SEQ ID NO: 1 - DNA, 24 bp, synthetic construct
  source 1..24: mol_type = other DNA
agctgagaccctgtatgcacagcc

SEQ ID NO: 2 - DNA, 23 bp, synthetic construct
  source 1..23: mol_type = other DNA
gcccacagcacccctgctattgt

SEQ ID NO: 3 - DNA, 30 bp, synthetic construct
  source 1..30: mol_type = other DNA
tgcattcaatcttcctgaactgcaaaagcc

SEQ ID NO: 4 - DNA, 35 bp, synthetic construct
  source 1..35: mol_type = other DNA
tggataaacaaggtccttctgtatagcacagagaa

SEQ ID NO: 5 - DNA, 21 bp, synthetic construct
  source 1..21: mol_type = other DNA
cccaggtgaaagtgacgtcct

SEQ ID NO: 6 - DNA, 21 bp, synthetic construct
  source 1..21: mol_type = other DNA
gtaaacggcgtactgcgtcca

SEQ ID NO: 7 - DNA, 25 bp, synthetic construct
  source 1..25: mol_type = other DNA
gaatcctctaacatgcattgccgtc

SEQ ID NO: 8 - DNA, 23 bp, synthetic construct
  source 1..23: mol_type = other DNA
ggcaagtggaacttttgagccca

SEQ ID NO: 9 - DNA, 25 bp, synthetic construct
  source 1..25: mol_type = other DNA
ttcttccattcaagaaccactgtcc

SEQ ID NO: 10 - DNA, 25 bp, synthetic construct
  source 1..25: mol_type = other DNA
cctacatgttcatttctggtcagca

SEQ ID NO: 11 - DNA, 21 bp, synthetic construct
  source 1..21: mol_type = other DNA
tcgaagggacacctggcagtt

SEQ ID NO: 12 - DNA, 24 bp, synthetic construct
  source 1..24: mol_type = other DNA
acaatggaaggtattgcttcccca

SEQ ID NO: 13 - DNA, 24 bp, synthetic construct
  source 1..24: mol_type = other DNA
tcacctttctctgcatgtccagtt

SEQ ID NO: 14 - DNA, 25 bp, synthetic construct
  source 1..25: mol_type = other DNA
ggaatttagatgacaagcaactgtt

SEQ ID NO: 15 - DNA, 22 bp, synthetic construct
  source 1..22: mol_type = other DNA
agtgaggaccaacacctgatgc

SEQ ID NO: 16 - DNA, 21 bp, synthetic construct
  source 1..21: mol_type = other DNA
ttttgcgcttgcagatccggt

SEQ ID NO: 17 - DNA, 25 bp, synthetic construct
  source 1..25: mol_type = other DNA
acatctgctaatacaccttacccgt

SEQ ID NO: 18 - DNA, 25 bp, synthetic construct
  source 1..25: mol_type = other DNA
ggaaaatcatttgcctctcagatgc

SEQ ID NO: 19 - DNA, 24 bp, synthetic construct
  source 1..24: mol_type = other DNA
actatagtggctctccagttcacc

SEQ ID NO: 20 - DNA, 25 bp, synthetic construct
  source 1..25: mol_type = other DNA
tcacatgcaatcttgaacatgccac

SEQ ID NO: 21 - DNA, 84 bp, synthetic construct
  source 1..84: mol_type = other DNA
tttttttttttttttttttttttttttttttttttttttttttttttttttttttttttcaggcagagcagggtgaaagccagg

SEQ ID NO: 22 - DNA, 78 bp, synthetic construct
  source 1..78: mol_type = other DNA
ttttttttttttttttttttttttttttttttttttttttttttttttttgcttacaaactctttgaaggtgtcagca

SEQ ID NO: 23 - DNA, 36 bp, synthetic construct
  source 1..36: mol_type = other DNA
ttttttttttggctgggatggtttcggagaagcaga

SEQ ID NO: 24 - DNA, 48 bp, synthetic construct
  source 1..48: mol_type = other DNA
ttttttttttttttttttttttttatctttggggcaaaggatgatgac

SEQ ID NO: 25 - DNA, 25 bp, synthetic construct
  source 1..25: mol_type = other DNA
cagctgttatgaacctgacattctg

SEQ ID NO: 26 - DNA, 30 bp, synthetic construct
  source 1..30: mol_type = other DNA
tttttttggcatctacctcgcagaagtaag

SEQ ID NO: 27 - DNA, 42 bp, synthetic construct
  source 1..42: mol_type = other DNA
tttttttttttttttttttgtgtaaccttatccttaaggaaa

SEQ ID NO: 28 - DNA, 108 bp, synthetic construct
  source 1..108: mol_type = other DNA
tttttttttttttttttttttttttttttttttttttttttttttttttttttttttttttttttttttttttttttttttttgctgtacatacctttctgcgctgaa

SEQ ID NO: 29 - DNA, 102 bp, synthetic construct
  source 1..102: mol_type = other DNA
ttttttttttttttttttttttttttttttttttttttttttttttttttttttttttttttttttttttttttttctcttgtgtcagggtgtggtctccac

SEQ ID NO: 30 - DNA, 108 bp, synthetic construct
  source 1..108: mol_type = other DNA
tttttttttttttttttttttttttttttttttttttttttttttttttttttttttttttttttttttttttttttttttttatgaaccctttgccctgggcatacc

SEQ ID NO: 31 - DNA, 66 bp, synthetic construct
  source 1..66: mol_type = other DNA
tttttttttttttttttttttttttttttttttttttttttagcgaagggctgtcacagctgcccc

SEQ ID NO: 32 - DNA, 30 bp, synthetic construct
  source 1..30: mol_type = other DNA
tttttggcgtcaaccttctcattttgtttt

SEQ ID NO: 33 - DNA, 90 bp, synthetic construct
  source 1..90: mol_type = other DNA
cccccccccccccccccccccccccccccccccccccccccccccccccccccccccccccccccgcaaccaggacgaggggtcatccca

SEQ ID NO: 34 - DNA, 66 bp, synthetic construct
  source 1..66: mol_type = other DNA
cccccccccccccccccccccccccccccccccccccccccgaatagaggaaggaagaaagagatt

SEQ ID NO: 35 - DNA, 96 bp, synthetic construct
  source 1..96: mol_type = other DNA
cccccccccccccccccccccccccccccccccccccccccccccccccccccccccccccccccccccccaaattgacccagcgtcctgcaggtc

SEQ ID NO: 36 - DNA, 42 bp, synthetic construct
  source 1..42: mol_type = other DNA
cccccccccccccccccgttgggcgggaggtccacgtccacc